European Patent Specification EP 3 688 155 B1, published January 4, 2023. Title: A UNIVERSAL PLATFORM FOR CAR THERAPY TARGETING A NOVEL ANTIGENIC SIGNATURE OF CANCER. Applicant: ImmPACT-Bio Ltd. Gavish-Galilee Bio Applications, Ltd. Gross, Gideon Gibson, Will Dahary, Dvir Beiman, Merav. The sequence listing filed with the application follows.

SEQUENCE LISTING (10 sequences)

SEQ ID NO: 1 - DNA, 3432 bp, Artificial Sequence
  CD19 aCAR_IRES_RFP_P2A_Puro Synthetic DNA
atggccttaccagtgaccgccttgctcctgccgctggccttgctgctccacgccgccaggccggacatccagatgacacagactacatcctccctgtctgcctctctgggagacagagtcaccatcagttgcagggcaagtcaggacattagtaaatatttaaattggtatcagcagaaaccagatggaactgttaaactcctgatctaccatacatcaagattacactcaggagtcccatcaaggttcagtggcagtgggtctggaacagattattctctcaccattagcaacctggagcaagaagatattgccacttacttttgccaacagggtaatacgcttccgtacacgttcggaggggggaccaagctggagatcacaggtggcggtggctcgggcggtggtgggtcgggtggcggcggatctgaggtgaaactgcaggagtcaggacctggcctggtggcgccctcacagagcctgtccgtcacatgcactgtctcaggggtctcattacccgactatggtgtaagctggattcgccagcctccacgaaagggtctggagtggctgggagtaatatggggtagtgaaaccacatactataattcagctctcaaatccagactgaccatcatcaaggacaactccaagagccaagttttcttaaaaatgaacagtctgcaaactgatgacacagccatttactactgtgccaaacattattactacggtggtagctatgctatggactactggggccaaggaacctcagtcaccgtctcctcaaccactaccccagcaccgaggccacccaccccggctcctaccatcgcctcccagcctctgtccctgcgtccggaggcatgtagacccgcagctggtggggccgtgcatacccggggtcttgacttcgcctgcgatatctacatttgggcccctctggctggtacttgcggggtcctgctgctttcactcgtgatcactctttactgtaagcgcggtcggaagaagctgctgtacatctttaagcaacccttcatgaggcctgtgcagactactcaagaggaggacggctgttcatgccggttcccagaggaggaggaaggcggctgcgaactgcgcgtgaaattcagccgcagcgcagatgctccagcctacaagcaggggcagaaccagctctacaacgaactcaatcttggtcggagagaggagtacgacgtgctggacaagcggagaggacgggacccagaaatgggcgggaagccgcgcagaaagaatccccaagagggcctgtacaacgagctccaaaaggataagatggcagaagcctatagcgagattggtatgaaaggggaacgcagaagaggcaaaggccacgacggactgtaccagggactcagcaccgccaccaaggacacctatgacgctcttcacatgcaggccctgccgcctcggtgagcggccgcaaattccgcccctctccctcccccccccctaacgttactggccgaagccgcttggaataaggccggtgtgcgtttgtctatatgttattttccaccatattgccgtcttttggcaatgtgagggcccggaaacctggccctgtcttcttgacgagcattcctaggggtctttcccctctcgccaaaggaatgcaaggtctgttgaatgtcgtgaaggaagcagttcctctggaagcttcttgaagacaaacaacgtctgtagcgaccctttgcaggcagcggaaccccccacctggcgacaggtgcctctgcggccaaaagccacgtgtataagatacacctgcaaaggcggcacaaccccagtgccacgttgtgagttggatagttgtggaaagagtcaaatggctctcctcaagcgtattcaacaaggggctgaaggatgcccagaaggtaccccattgtatgggatctgatctggggcctcggtgcacatgctttacatgtgtttagtcgaggttaaaaaaacgtctaggccccccgaaccacggggacgtggttttcctttgaaaaacacgataataccatggtgtctaagggcgaagagctgattaaggagaacatgcacatgaagctgtacatggagggcaccgtgaacaaccaccacttcaagtgcacatccgagggcgaaggcaagccctacgagggcacccagaccatgagaatcaaggtggtcgagggcggccctctccccttcgccttcgacatcctggctaccagcttcatgtacggcagcagaaccttcatcaaccacacccagggcatccccgacttctttaagcagtccttccctgagggcttcacatgggagagagtcaccacatacgaagacgggggcgtgctgaccgctacccaggacaccagcctccaggacggctgcctcatctacaacgtcaagatcagaggggtgaacttcccatccaacggccctgtgatgcagaagaaaacactcggctgggaggccaacaccgagatgctgtaccccgctgacggcggcctggaaggcagaagcgacatggccctgaagctcgtgggcgggggccacctgatctgcaacttcaagaccacatacagatccaagaaacccgctaagaacctcaagatgcccggcgtctactatgtggaccacagactggaaagaatcaaggaggccgacaaagagacctacgtcgagcagcacgaggtggctgtggccagatactgcgacctccctagcaaactggggcacaaacttaatggatccggcgcgacaaactttagcttgctgaagcaagctggtgacgtggaggagaatcccggccctatggccaccgagtacaagcccacggtgcgcctcgccacccgcgacgacgtcccccgggccgtacgcaccctcgccgccgcgttcgccgactaccccgccacgcgccacaccgtcgatccggaccgccacatcgagcgggtcaccgagctgcaagaactcttcctcacgcgcgtcgggctcgacatcggcaaggtgtgggtcgcggacgacggcgccgcggtggcggtctggaccacgccggagagcgtcgaagcgggggcggtgttcgccgagatcggcccgcgcatggccgagttgagcggttcccggctggccgcgcagcaacagatggaaggcctcctggcgccgcaccggcccaaggagcccgcgtggttcctggccaccgtcggcgtctcgcccgaccaccagggcaagggtctgggcagcgccgtcgtgctccccggagtggaggcggccgagcgcgccggggtgcccgccttcctggagacctccgcgccccgcaacctccccttctacgagcggctcggcttcaccgtcaccgccgacgtcgaggtgcccgaaggaccgcgcacctggtgcatgacccgcaagcccggtgcctga

SEQ ID NO: 2 - protein, 486 aa, Artificial Sequence
  CD19 aCAR Synthetic protein
MALPVTALLLPLALLLHAARPDIQMTQTTSSLSASLGDRVTISCRASQDISKYLNWYQQKPDGTVKLLIYHTSRLHSGVPSRFSGSGSGTDYSLTISNLEQEDIATYFCQQGNTLPYTFGGGTKLEITGGGGSGGGGSGGGGSEVKLQESGPGLVAPSQSLSVTCTVSGVSLPDYGVSWIRQPPRKGLEWLGVIWGSETTYYNSALKSRLTIIKDNSKSQVFLKMNSLQTDDTAIYYCAKHYYYGGSYAMDYWGQGTSVTVSSTTTPAPRPPTPAPTIASQPLSLRPEACRPAAGGAVHTRGLDFACDIYIWAPLAGTCGVLLLSLVITLYCKRGRKKLLYIFKQPFMRPVQTTQEEDGCSCRFPEEEEGGCELRVKFSRSADAPAYKQGQNQLYNELNLGRREEYDVLDKRRGRDPEMGGKPRRKNPQEGLYNELQKDKMAEAYSEIGMKGERRRGKGHDGLYQGLSTATKDTYDALHMQALPPR

SEQ ID NO: 3 - protein, 237 aa, Artificial Sequence
  RFP Synthetic Protein
MVSKGEELIKENMHMKLYMEGTVNNHHFKCTSEGEGKPYEGTQTMRIKVVEGGPLPFAFDILATSFMYGSRTFINHTQGIPDFFKQSFPEGFTWERVTTYEDGGVLTATQDTSLQDGCLIYNVKIRGVNFPSNGPVMQKKTLGWEANTEMLYPADGGLEGRSDMALKLVGGGHLICNFKTTYRSKKPAKNLKMPGVYYVDHRLERIKEADKETYVEQHEVAVARYCDLPSKLGHKLN

SEQ ID NO: 4 - protein, 200 aa, Artificial Sequence
  Puromycin resistance Synthetic Protein
MATEYKPTVRLATRDDVPRAVRTLAAAFADYPATRHTVDPDRHIERVTELQELFLTRVGLDIGKVWVADDGAAVAVWTTPESVEAGAVFAEIGPRMAELSGSRLAAQQQMEGLLAPHRPKEPAWFLATVGVSPDHQGKGLGSAVVLPGVEAAERAGVPAFLETSAPRNLPFYERLGFTVTADVEVPEGPRTWCMTRKPGA

SEQ ID NO: 5 - DNA, 3669 bp, Artificial Sequence
  CD20 iCAR_IRES_GFP_P2A_Hygro Synthetic DNA
atggcactgcctgtgaccgccctgctgctgccactggccctgctgctgcacgcagccaggcccgacatcgtgctgacacagagcccagcaatcctgtccgcctctcctggagagaaggtgaccatgacatgccgcgccagctcctctgtgaactacatggattggtatcagaagaagcctggcagctccccaaagccctggatctacgccaccagcaatctggcctccggcgtgccagcacggttcagcggctccggctctggcaccagctattccctgacaatctccagagtggaggcagaggacgcagcaacctactattgccagcagtggtctttcaacccccctacctttggcggcggcacaaagctggagatcaagggctctacaagcggaggaggctctggaggaggcagcggaggcggcggctctagcgaggtgcagctgcagcagagcggagcagagctggtgaagcctggagcctccgtgaagatgtcttgtaaggccagcggctacaccttcacatcctataatatgcactgggtgaagcagaccccaggacagggcctggagtggatcggagcaatctacccaggaaacggcgacacaagctataatcagaagtttaagggcaaggccaccctgacagccgataagtcctctagcaccgcctacatgcagctgtcctctctgacatccgaggactctgccgattactattgtgcccggtccaactactatggcagctcctactggttctttgacgtgtggggagcaggcaccacagtgaccgtgtctagcaccgagaggagagcagaggtgcccacagcacacccatctccaagccctaggccagcaggacagttccagaccctggtggtgggagtggtgggaggcctgctgggctctctggtgctgctggtgtgggtgctggccgtgatctgcagcagggccgcccgcggcaccatcggcgccaggcgcacaggccagcctctgaaggaggacccttccgccgtgccagtgttctctgtggactacggcgagctggattttcagtggcgggagaaaaccccagagccacctgtgccctgcgtgcctgagcagaccgagtatgccacaatcgtgtttccatccggaatgggcacaagctcccctgcaaggagaggcagcgccgacggaccacggtccgcccagccactgcggcccgaggatggccactgttcttggcccctgtgacgcccctctcccccccccccctctccctcccccccccctaacgttactggccgaagccgcttggaataaggccggtgtgcgtttgtctatatgttattttccaccatattgccgtcttttggcaatgtgagggcccggaaacctggccctgtcttcttgacgagcattcctaggggtctttcccctctcgccaaaggaatgcaaggtctgttgaatgtcgtgaaggaagcagttcctctggaagcttcttgaagacaaacaacgtctgtagcgaccctttgcaggcagcggaaccccccacctggcgacaggtgcctctgcggccaaaagccacgtgtataagatacacctgcaaaggcggcacaaccccagtgccacgttgtgagttggatagttgtggaaagagtcaaatggctctcctcaagcgtattcaacaaggggctgaaggatgcccagaaggtaccccattgtatgggatctgatctggggcctcggtgcacatgctttacatgtgtttagtcgaggttaaaaaaacgtctaggccccccgaaccacggggacgtggttttcctttgaaaaacacgatgataaggcttgccacaacccgtaccaaagatggtgtccaagggagaggagctgttcaccggagtggtgcccatcctggtggagctggacggcgatgtgaatggccacaagtttagcgtgtccggagagggagagggcgacgcaacctacggcaagctgacactgaagttcatctgcaccacaggcaagctgcccgtgccttggccaaccctggtgaccacactgacatacggcgtgcagtgtttttctcgctatcccgaccacatgaagcagcacgatttctttaagagcgccatgcctgagggctacgtgcaggagcggaccatcttctttaaggacgatggcaactataagaccagagccgaggtgaagttcgagggcgacacactggtgaacaggatcgagctgaagggcatcgactttaaggaggatggcaatatcctgggccacaagctggagtacaactataattcccacaacgtgtacatcatggccgataagcagaagaacggcatcaaggtcaatttcaagatcagacacaatatcgaggacggctctgtgcagctggccgatcactaccagcagaacaccccaatcggcgacggacccgtgctgctgcctgataatcactatctgtctacacagagcgccctgtccaaggaccccaacgagaagagggatcacatggtgctgctggagtttgtgaccgcagcaggaatcacactgggaatggacgagctgtataagggcagcggcgccaccaacttctccctgctgaagcaggcaggcgacgtggaggagaatccaggacctatggatagaagcggcaagccagagctgaccgccacatccgtggagaagttcctgatcgagaagtttgactctgtgagcgatctgatgcagctgtccgagggagaggagtccagggccttctcttttgatgtgggcggcaggggatacgtgctgagggtgaatagctgcgccgacggcttctataaggatagatacgtgtatagacactttgcctccgccgccctgccaatcccagaggtgctggacatcggcgagttttccgagtctctgacctactgtatcagccggagagcccagggagtgaccctgcaggatctgcctgagacagagctgccagccgtgctgcagccagtggcagaggctatggacgcaatcgccgccgccgacctgtctcagacaagcggcttcggcccttttggcccacagggcatcggccagtacaccacatggagggacttcatctgcgccatcgccgatcctcacgtgtatcactggcagaccgtgatggacgatacagtgagcgcctccgtggcacaggccctggacgagctgatgctgtgggccgaggattgtccagaggtgcgccacctggtgcacgcagactttggcagcaacaatgtgctgaccgataatggccggatcacagccgtgatcgactggtccgaggccatgttcggcgattctcagtacgaggtggccaacatcttcttttggaggccttggctggcctgcatggagcagcagacccgctattttgagaggcgccaccctgagctggccggctctccacggctgagagcatacatgctgcgcatcggcctggaccagctgtatcagagcctggtggatggcaatttcgacgatgcagcatgggcacagggccggtgcgacgcaatcgtgagatccggcgccggcaccgtgggccggacacagatcgcacggcggagcgccgccgtgtggaccgacggatgcgtggaggtgctggccgattctggcaacaggcgcccaagcacaaggccccgcgccaaggagtga

SEQ ID NO: 6 - protein, 411 aa, Artificial Sequence
  CD20 iCAR Synthetic Protein
MALPVTALLLPLALLLHAARPDIVLTQSPAILSASPGEKVTMTCRASSSVNYMDWYQKKPGSSPKPWIYATSNLASGVPARFSGSGSGTSYSLTISRVEAEDAATYYCQQWSFNPPTFGGGTKLEIKGSTSGGGSGGGSGGGGSSEVQLQQSGAELVKPGASVKMSCKASGYTFTSYNMHWVKQTPGQGLEWIGAIYPGNGDTSYNQKFKGKATLTADKSSSTAYMQLSSLTSEDSADYYCARSNYYGSSYWFFDVWGAGTTVTVSSTERRAEVPTAHPSPSPRPAGQFQTLVVGVVGGLLGSLVLLVWVLAVICSRAARGTIGARRTGQPLKEDPSAVPVFSVDYGELDFQWREKTPEPPVPCVPEQTEYATIVFPSGMGTSSPARRGSADGPRSAQPLRPEDGHCSWPL

SEQ ID NO: 7 - protein, 239 aa, Artificial Sequence
  GFP Synthetic Protein
MVSKGEELFTGVVPILVELDGDVNGHKFSVSGEGEGDATYGKLTLKFICTTGKLPVPWPTLVTTLTYGVQCFSRYPDHMKQHDFFKSAMPEGYVQERTIFFKDDGNYKTRAEVKFEGDTLVNRIELKGIDFKEDGNILGHKLEYNYNSHNVYIMADKQKNGIKVNFKIRHNIEDGSVQLADHYQQNTPIGDGPVLLPDNHYLSTQSALSKDPNEKRDHMVLLEFVTAAGITLGMDELYK

SEQ ID NO: 8 - protein, 344 aa, Artificial Sequence
  Hygromycin resistance Synthetic Protein
MDRSGKPELTATSVEKFLIEKFDSVSDLMQLSEGEESRAFSFDVGGRGYVLRVNSCADGFYKDRYVYRHFASAALPIPEVLDIGEFSESLTYCISRRAQGVTLQDLPETELPAVLQPVAEAMDAIAAADLSQTSGFGPFGPQGIGQYTTWRDFICAIADPHVYHWQTVMDDTVSASVAQALDELMLWAEDCPEVRHLVHADFGSNNVLTDNGRITAVIDWSEAMFGDSQYEVANIFFWRPWLACMEQQTRYFERRHPELAGSPRLRAYMLRIGLDQLYQSLVDGNFDDAAWAQGRCDAIVRSGAGTVGRTQIARRSAAVWTDGCVEVLADSGNRRPSTRPRAKE

SEQ ID NO: 9 - DNA, 3696 bp, Artificial Sequence
  HLA-A2 iCAR_IRES_ GFP_P2A_Hygro Synthetic DNA
atggcactgccagtgaccgccctgctgctgcctctggccctgctgctgcacgcagccagacccgagcagaagctgatctccgaggaggacctgcaggtgcagctgcagcagtctggacctgagctggtgaagccaggagcctccgtgaagatgtcttgcaaggccagcggctacaccttcacatcttatcacatccagtgggtgaagcagcggcccggacagggcctggagtggatcggatggatctacccaggcgacggctccacacagtataacgagaagttcaagggcaagaccacactgaccgccgataagagcagcagcaccgcctacatgctgctgagcagcctgaccagcgaggacagcgccatctacttttgcgccagggagggcacatactatgctatggactattggggccagggcaccagcgtgacagtgtctagcggaggaggaggctccggaggaggaggctctggcggcggcggcagcgacgtgctgatgacccagacaccactgagcctgcccgtgagcctgggcgatcaggtgagcatctcctgtagatcctctcagagcatcgtgcactccaacggcaatacctacctggagtggtatctgcagaagccaggccagtcccccaagctgctgatctataaggtgtctaatcggttcagcggcgtgcctgacagattttctggcagcggctccggcaccgacttcaccctgaagatcagccgggtggaggcagaggatctgggcgtgtactattgtttccagggctcccacgtgccacgcacctttggcggcggcacaaagctggagatcaagaccgagaggagagcagaggtgcccacagcacacccatctccaagccctaggccagcaggacagttccagaccctggtggtgggagtggtgggaggcctgctgggctctctggtgctgctggtgtgggtgctggccgtgatctgcagcagggccgcccgcggcaccatcggcgccaggcgcacaggccagcctctgaaggaggacccttccgccgtgccagtgttctctgtggactacggcgagctggattttcagtggcgggagaaaaccccagagccacctgtgccctgcgtgcctgagcagaccgagtatgccacaatcgtgtttccatccggaatgggcacaagctcccctgcaaggagaggcagcgccgacggaccacggtccgcccagccactgcggcccgaggatggccactgttcttggcccctgtgacgcccctctcccccccccccctctccctcccccccccctaacgttactggccgaagccgcttggaataaggccggtgtgcgtttgtctatatgttattttccaccatattgccgtcttttggcaatgtgagggcccggaaacctggccctgtcttcttgacgagcattcctaggggtctttcccctctcgccaaaggaatgcaaggtctgttgaatgtcgtgaaggaagcagttcctctggaagcttcttgaagacaaacaacgtctgtagcgaccctttgcaggcagcggaaccccccacctggcgacaggtgcctctgcggccaaaagccacgtgtataagatacacctgcaaaggcggcacaaccccagtgccacgttgtgagttggatagttgtggaaagagtcaaatggctctcctcaagcgtattcaacaaggggctgaaggatgcccagaaggtaccccattgtatgggatctgatctggggcctcggtgcacatgctttacatgtgtttagtcgaggttaaaaaaacgtctaggccccccgaaccacggggacgtggttttcctttgaaaaacacgatgataaggcttgccacaacccgtaccaaagatggtgtccaagggagaggagctgttcaccggagtggtgcccatcctggtggagctggacggcgatgtgaatggccacaagtttagcgtgtccggagagggagagggcgacgcaacctacggcaagctgacactgaagttcatctgcaccacaggcaagctgcccgtgccttggccaaccctggtgaccacactgacatacggcgtgcagtgtttttctcgctatcccgaccacatgaagcagcacgatttctttaagagcgccatgcctgagggctacgtgcaggagcggaccatcttctttaaggacgatggcaactataagaccagagccgaggtgaagttcgagggcgacacactggtgaacaggatcgagctgaagggcatcgactttaaggaggatggcaatatcctgggccacaagctggagtacaactataattcccacaacgtgtacatcatggccgataagcagaagaacggcatcaaggtcaatttcaagatcagacacaatatcgaggacggctctgtgcagctggccgatcactaccagcagaacaccccaatcggcgacggacccgtgctgctgcctgataatcactatctgtctacacagagcgccctgtccaaggaccccaacgagaagagggatcacatggtgctgctggagtttgtgaccgcagcaggaatcacactgggaatggacgagctgtataagggcagcggcgccaccaacttctccctgctgaagcaggcaggcgacgtggaggagaatccaggacctatggatagaagcggcaagccagagctgaccgccacatccgtggagaagttcctgatcgagaagtttgactctgtgagcgatctgatgcagctgtccgagggagaggagtccagggccttctcttttgatgtgggcggcaggggatacgtgctgagggtgaatagctgcgccgacggcttctataaggatagatacgtgtatagacactttgcctccgccgccctgccaatcccagaggtgctggacatcggcgagttttccgagtctctgacctactgtatcagccggagagcccagggagtgaccctgcaggatctgcctgagacagagctgccagccgtgctgcagccagtggcagaggctatggacgcaatcgccgccgccgacctgtctcagacaagcggcttcggcccttttggcccacagggcatcggccagtacaccacatggagggacttcatctgcgccatcgccgatcctcacgtgtatcactggcagaccgtgatggacgatacagtgagcgcctccgtggcacaggccctggacgagctgatgctgtgggccgaggattgtccagaggtgcgccacctggtgcacgcagactttggcagcaacaatgtgctgaccgataatggccggatcacagccgtgatcgactggtccgaggccatgttcggcgattctcagtacgaggtggccaacatcttcttttggaggccttggctggcctgcatggagcagcagacccgctattttgagaggcgccaccctgagctggccggctctccacggctgagagcatacatgctgcgcatcggcctggaccagctgtatcagagcctggtggatggcaatttcgacgatgcagcatgggcacagggccggtgcgacgcaatcgtgagatccggcgccggcaccgtgggccggacacagatcgcacggcggagcgccgccgtgtggaccgacggatgcgtggaggtgctggccgattctggcaacaggcgcccaagcacaaggccccgcgccaaggagtga

SEQ ID NO: 10 - protein, 420 aa, Artificial Sequence
  HLA-A2 iCAR Synthetic Protein
MALPVTALLLPLALLLHAARPEQKLISEEDLQVQLQQSGPELVKPGASVKMSCKASGYTFTSYHIQWVKQRPGQGLEWIGWIYPGDGSTQYNEKFKGKTTLTADKSSSTAYMLLSSLTSEDSAIYFCAREGTYYAMDYWGQGTSVTVSSGGGGSGGGGSGGGGSDVLMTQTPLSLPVSLGDQVSISCRSSQSIVHSNGNTYLEWYLQKPGQSPKLLIYKVSNRFSGVPDRFSGSGSGTDFTLKISRVEAEDLGVYYCFQGSHVPRTFGGGTKLEIKTERRAEVPTAHPSPSPRPAGQFQTLVVGVVGGLLGSLVLLVWVLAVICSRAARGTIGARRTGQPLKEDPSAVPVFSVDYGELDFQWREKTPEPPVPCVPEQTEYATIVFPSGMGTSSPARRGSADGPRSAQPLRPEDGHCSWPL